European Patent Application EP 4 428 147 A2, published September 11, 2024. Title: ACTIVIN RECEPTOR TYPE IIA VARIANTS AND METHODS OF USE THEREOF. Applicant: KEROS THERAPEUTICS, INC. Application EP 24177118.7, filed November 9, 2018. The sequence listing filed with the application follows.

SEQUENCE LISTING (161 sequences)

SEQ ID NO: 1 - protein, 109 aa, synthetic construct
  source 1..109: note = Synthetic Construct
  VARIANT 14: note = MISC_FEATURE - Xaa is Phe or Tyr
  VARIANT 15: note = MISC_FEATURE - Xaa is Phe or Tyr
  VARIANT 20: note = MISC_FEATURE - Xaa is Glu or Ala
  VARIANT 21: note = MISC_FEATURE - Xaa is Lys or Leu
  VARIANT 22: note = MISC_FEATURE - Xaa is Asp or Glu
  VARIANT 23: note = MISC_FEATURE - Xaa is Arg or Ala
  VARIANT 31: note = MISC_FEATURE - Xaa is Pro or Arg
  VARIANT 33: note = MISC_FEATURE - Xaa is Tyr or Glu
  VARIANT 35: note = MISC_FEATURE - Xaa is Asp or Glu
  VARIANT 36: note = MISC_FEATURE - Xaa is Lys or Gln
  VARIANT 37: note = MISC_FEATURE - Xaa is Asp or Ala
  VARIANT 38: note = MISC_FEATURE - Xaa is Lys or Ala
  VARIANT 39: note = MISC_FEATURE - Xaa is Arg or Ala
  VARIANT 40: note = MISC_FEATURE - Xaa is Arg or Leu
  VARIANT 43: note = MISC_FEATURE - Xaa is Phe or Tyr
  VARIANT 47: note = MISC_FEATURE - Xaa is Lys, Arg, or Ala
  VARIANT 57: note = MISC_FEATURE - Xaa is Lys, Ala, Tyr, Phe, or Ile
  VARIANT 58: note = MISC_FEATURE - Xaa is Gln or Lys
  VARIANT 61: note = MISC_FEATURE - Xaa is Trp or Ala
  VARIANT 62: note = MISC_FEATURE - Xaa is Leu or Ala
  VARIANT 63: note = MISC_FEATURE - Xaa is Asp, Lys, Arg, Ala, Phe, Gly, Met, Asn, or Ile
  VARIANT 65: note = MISC_FEATURE - Xaa is Ile, Phe, or Ala
  VARIANT 76: note = MISC_FEATURE - Xaa is Lys or Thr
  VARIANT 77: note = MISC_FEATURE - Xaa is Lys or Glu
  VARIANT 78: note = MISC_FEATURE - Xaa is Asp or Glu
  VARIANT 79: note = MISC_FEATURE - Xaa is Ser or Asn
  VARIANT 81: note = MISC_FEATURE - Xaa is Glu or Gln
GAILGRSETQECLXXNANWXXXXTNQTGVEXCXGXXXXXXHCXATWXNISGSIEIVXXGCXXXDXNCYDRTDCVEXXXXPXVYFCCCEGNMCNEKFSYFPEMEVTQPTS

SEQ ID NO: 2 - protein, 109 aa, synthetic construct
  source 1..109: note = Synthetic Construct
  VARIANT 15: note = MISC_FEATURE - Xaa is Phe or Tyr
  VARIANT 20: note = MISC_FEATURE - Xaa is Glu or Ala
  VARIANT 21: note = MISC_FEATURE - Xaa is Lys or Leu
  VARIANT 22: note = MISC_FEATURE - Xaa is Asp or Glu
  VARIANT 23: note = MISC_FEATURE - Xaa is Arg or Ala
  VARIANT 31: note = MISC_FEATURE - Xaa is Pro or Arg
  VARIANT 33: note = MISC_FEATURE - Xaa is Tyr or Glu
  VARIANT 35: note = MISC_FEATURE - Xaa is Asp or Glu
  VARIANT 37: note = MISC_FEATURE - Xaa is Asp or Ala
  VARIANT 38: note = MISC_FEATURE - Xaa is Lys or Ala
  VARIANT 39: note = MISC_FEATURE - Xaa is Arg or Ala
  VARIANT 40: note = MISC_FEATURE - Xaa is Arg or Leu
  VARIANT 43: note = MISC_FEATURE - Xaa is Phe or Tyr
  VARIANT 47: note = MISC_FEATURE - Xaa is Lys, Arg, or Ala
  VARIANT 57: note = MISC_FEATURE - Xaa is Lys, Ala, Tyr, Phe, or Ile
  VARIANT 58: note = MISC_FEATURE - Xaa is Gln or Lys
  VARIANT 61: note = MISC_FEATURE - Xaa is Trp or Ala
  VARIANT 62: note = MISC_FEATURE - Xaa is Leu or Ala
  VARIANT 63: note = MISC_FEATURE - Xaa is Asp, Lys, Arg, Ala, Phe, Gly, Met, Asn, or Ile
  VARIANT 65: note = MISC_FEATURE - Xaa is Ile, Phe, or Ala
  VARIANT 76: note = MISC_FEATURE - Xaa is Lys or Thr
  VARIANT 77: note = MISC_FEATURE - Xaa is Lys or Glu
  VARIANT 78: note = MISC_FEATURE - Xaa is Asp or Glu
  VARIANT 79: note = MISC_FEATURE - Xaa is Ser or Asn
  VARIANT 81: note = MISC_FEATURE - Xaa is Glu or Gln
GAILGRSETQECLFXNANWXXXXTNQTGVEXCXGXKXXXXHCXATWXNISGSIEIVXXGCXXXDXNCYDRTDCVEXXXXPXVYFCCCEGNMCNEKFSYFPEMEVTQPTS

SEQ ID NO: 3 - protein, 109 aa, synthetic construct
  source 1..109: note = Synthetic Construct
  VARIANT 15: note = MISC_FEATURE - Xaa is Phe or Tyr
  VARIANT 21: note = MISC_FEATURE - Xaa is Lys or Leu
  VARIANT 22: note = MISC_FEATURE - Xaa is Asp or Glu
  VARIANT 31: note = MISC_FEATURE - Xaa is Pro or Arg
  VARIANT 33: note = MISC_FEATURE - Xaa is Tyr or Glu
  VARIANT 35: note = MISC_FEATURE - Xaa is Asp or Glu
  VARIANT 40: note = MISC_FEATURE - Xaa is Arg or Leu
  VARIANT 43: note = MISC_FEATURE - Xaa is Phe or Tyr
  VARIANT 47: note = MISC_FEATURE - Xaa is Lys, Arg, or Ala
  VARIANT 58: note = MISC_FEATURE - Xaa is Gln or Lys
  VARIANT 65: note = MISC_FEATURE - Xaa is Ile, Phe, or Ala
  VARIANT 76: note = MISC_FEATURE - Xaa is Lys or Thr
  VARIANT 77: note = MISC_FEATURE - Xaa is Lys or Glu
  VARIANT 78: note = MISC_FEATURE - Xaa is Asp or Glu
  VARIANT 79: note = MISC_FEATURE - Xaa is Ser or Asn
  VARIANT 81: note = MISC_FEATURE - Xaa is Glu or Gln
GAILGRSETQECLFXNANWEXXRTNQTGVEXCXGXKDKRXHCXATWXNISGSIEIVKXGCWLDDXNCYDRTDCVEXXXXPXVYFCCCEGNMCNEKFSYFPEMEVTQPTS

SEQ ID NO: 4 - protein, 109 aa, synthetic construct
  source 1..109: note = Synthetic Construct
  VARIANT 15: note = MISC_FEATURE - Xaa is Phe or Tyr
  VARIANT 21: note = MISC_FEATURE - Xaa is Lys or Leu
  VARIANT 31: note = MISC_FEATURE - Xaa is Pro or Arg
  VARIANT 33: note = MISC_FEATURE - Xaa is Tyr or Glu
  VARIANT 35: note = MISC_FEATURE - Xaa is Asp or Glu
  VARIANT 40: note = MISC_FEATURE - Xaa is Arg or Leu
  VARIANT 43: note = MISC_FEATURE - Xaa is Phe or Tyr
  VARIANT 47: note = MISC_FEATURE - Xaa is Lys, Arg, or Ala
  VARIANT 58: note = MISC_FEATURE - Xaa is Gln or Lys
  VARIANT 65: note = MISC_FEATURE - Xaa is Ile, Phe, or Ala
  VARIANT 76: note = MISC_FEATURE - Xaa is Lys or Thr
  VARIANT 78: note = MISC_FEATURE - Xaa is Asp or Glu
  VARIANT 79: note = MISC_FEATURE - Xaa is Ser or Asn
  VARIANT 81: note = MISC_FEATURE - Xaa is Glu or Gln
GAILGRSETQECLFXNANWEXDRTNQTGVEXCXGXKDKRXHCXATWXNISGSIEIVKXGCWLDDXNCYDRTDCVEXKXXPXVYFCCCEGNMCNEKFSYFPEMEVTQPTS

SEQ ID NO: 5 - protein, 109 aa, synthetic construct
  source 1..109: note = Synthetic Construct
  VARIANT 15: note = MISC_FEATURE - Xaa is Phe or Tyr
  VARIANT 21: note = MISC_FEATURE - Xaa is Lys or Leu
  VARIANT 33: note = MISC_FEATURE - Xaa is Tyr or Glu
  VARIANT 35: note = MISC_FEATURE - Xaa is Asp or Glu
  VARIANT 40: note = MISC_FEATURE - Xaa is Arg or Leu
  VARIANT 58: note = MISC_FEATURE - Xaa is Gln or Lys
  VARIANT 76: note = MISC_FEATURE - Xaa is Lys or Thr
  VARIANT 78: note = MISC_FEATURE - Xaa is Asp or Glu
  VARIANT 79: note = MISC_FEATURE - Xaa is Ser or Asn
  VARIANT 81: note = MISC_FEATURE - Xaa is Glu or Gln
GAILGRSETQECLFXNANWEXDRTNQTGVEPCXGXKDKRXHCFATWKNISGSIEIVKXGCWLDDINCYDRTDCVEXKXXPXVYFCCCEGNMCNEKFSYFPEMEVTQPTS

SEQ ID NO: 6 - protein, 109 aa, synthetic construct
  source 1..109: note = Synthetic Construct
GAILGRSETQECLFYNANWELDRTNQTGVEPCEGEKDKRLHCFATWKNISGSIEIVKKGCWLDDINCYDRTDCVETKENPQVYFCCCEGNMCNEKFSYFPEMEVTQPTS

SEQ ID NO: 7 - protein, 109 aa, synthetic construct
  source 1..109: note = Synthetic Construct
GAILGRSETQECLFYNANWELERTNQTGVEPCEGEKDKRLHCFATWKNISGSIEIVKKGCWLDDINCYDRTDCVETKENPQVYFCCCEGNMCNEKFSYFPEMEVTQPTS

SEQ ID NO: 8 - protein, 109 aa, synthetic construct
  source 1..109: note = Synthetic Construct
GAILGRSETQECLFYNANWELDRTNQTGVERCEGEKDKRLHCFATWKNISGSIEIVKKGCWLDDINCYDRTDCVETKENPQVYFCCCEGNMCNEKFSYFPEMEVTQPTS

SEQ ID NO: 9 - protein, 109 aa, synthetic construct
  source 1..109: note = Synthetic Construct
GAILGRSETQECLFYNANWELDRTNQTGVEPCEGEKDKRLHCYATWKNISGSIEIVKKGCWLDDINCYDRTDCVETKENPQVYFCCCEGNMCNEKFSYFPEMEVTQPTS

SEQ ID NO: 10 - protein, 109 aa, synthetic construct
  source 1..109: note = Synthetic Construct
GAILGRSETQECLFYNANWELDRTNQTGVEPCEGEKDKRLHCFATWRNISGSIEIVKKGCWLDDINCYDRTDCVETKENPQVYFCCCEGNMCNEKFSYFPEMEVTQPTS

SEQ ID NO: 11 - protein, 109 aa, synthetic construct
  source 1..109: note = Synthetic Construct
GAILGRSETQECLFYNANWELDRTNQTGVEPCEGEKDKRLHCFATWKNISGSIEIVKKGCWLDDFNCYDRTDCVETKENPQVYFCCCEGNMCNEKFSYFPEMEVTQPTS

SEQ ID NO: 12 - protein, 109 aa, synthetic construct
  source 1..109: note = Synthetic Construct
GAILGRSETQECLFYNANWELDRTNQTGVEPCEGEKDKRLHCFATWKNISGSIEIVKKGCWLDDINCYDRTDCVETEENPQVYFCCCEGNMCNEKFSYFPEMEVTQPTS

SEQ ID NO: 13 - protein, 109 aa, synthetic construct
  source 1..109: note = Synthetic Construct
GAILGRSETQECLFYNANWELERTNQTGVERCEGEKDKRLHCFATWKNISGSIEIVKKGCWLDDINCYDRTDCVETKENPQVYFCCCEGNMCNEKFSYFPEMEVTQPTS

SEQ ID NO: 14 - protein, 109 aa, synthetic construct
  source 1..109: note = Synthetic Construct
GAILGRSETQECLFYNANWELERTNQTGVEPCEGEKDKRLHCYATWKNISGSIEIVKKGCWLDDINCYDRTDCVETKENPQVYFCCCEGNMCNEKFSYFPEMEVTQPTS

SEQ ID NO: 15 - protein, 109 aa, synthetic construct
  source 1..109: note = Synthetic Construct
GAILGRSETQECLFYNANWELERTNQTGVEPCEGEKDKRLHCFATWRNISGSIEIVKKGCWLDDINCYDRTDCVETKENPQVYFCCCEGNMCNEKFSYFPEMEVTQPTS

SEQ ID NO: 16 - protein, 109 aa, synthetic construct
  source 1..109: note = Synthetic Construct
GAILGRSETQECLFYNANWELERTNQTGVEPCEGEKDKRLHCFATWKNISGSIEIVKKGCWLDDFNCYDRTDCVETKENPQVYFCCCEGNMCNEKFSYFPEMEVTQPTS

SEQ ID NO: 17 - protein, 109 aa, synthetic construct
  source 1..109: note = Synthetic Construct
GAILGRSETQECLFYNANWELERTNQTGVEPCEGEKDKRLHCFATWKNISGSIEIVKKGCWLDDINCYDRTDCVETEENPQVYFCCCEGNMCNEKFSYFPEMEVTQPTS

SEQ ID NO: 18 - protein, 109 aa, synthetic construct
  source 1..109: note = Synthetic Construct
GAILGRSETQECLFYNANWELDRTNQTGVERCEGEKDKRLHCYATWKNISGSIEIVKKGCWLDDINCYDRTDCVETKENPQVYFCCCEGNMCNEKFSYFPEMEVTQPTS

SEQ ID NO: 19 - protein, 109 aa, synthetic construct
  source 1..109: note = Synthetic Construct
GAILGRSETQECLFYNANWELDRTNQTGVERCEGEKDKRLHCFATWRNISGSIEIVKKGCWLDDINCYDRTDCVETKENPQVYFCCCEGNMCNEKFSYFPEMEVTQPTS

SEQ ID NO: 20 - protein, 109 aa, synthetic construct
  source 1..109: note = Synthetic Construct
GAILGRSETQECLFYNANWELDRTNQTGVERCEGEKDKRLHCFATWKNISGSIEIVKKGCWLDDFNCYDRTDCVETKENPQVYFCCCEGNMCNEKFSYFPEMEVTQPTS

SEQ ID NO: 21 - protein, 109 aa, synthetic construct
  source 1..109: note = Synthetic Construct
GAILGRSETQECLFYNANWELDRTNQTGVERCEGEKDKRLHCFATWKNISGSIEIVKKGCWLDDINCYDRTDCVETEENPQVYFCCCEGNMCNEKFSYFPEMEVTQPTS

SEQ ID NO: 22 - protein, 109 aa, synthetic construct
  source 1..109: note = Synthetic Construct
GAILGRSETQECLFYNANWELDRTNQTGVEPCEGEKDKRLHCYATWRNISGSIEIVKKGCWLDDINCYDRTDCVETKENPQVYFCCCEGNMCNEKFSYFPEMEVTQPTS

SEQ ID NO: 23 - protein, 109 aa, synthetic construct
  source 1..109: note = Synthetic Construct
GAILGRSETQECLFYNANWELDRTNQTGVEPCEGEKDKRLHCYATWKNISGSIEIVKKGCWLDDFNCYDRTDCVETKENPQVYFCCCEGNMCNEKFSYFPEMEVTQPTS

SEQ ID NO: 24 - protein, 109 aa, synthetic construct
  source 1..109: note = Synthetic Construct
GAILGRSETQECLFYNANWELDRTNQTGVEPCEGEKDKRLHCYATWKNISGSIEIVKKGCWLDDINCYDRTDCVETEENPQVYFCCCEGNMCNEKFSYFPEMEVTQPTS

SEQ ID NO: 25 - protein, 109 aa, synthetic construct
  source 1..109: note = Synthetic Construct
GAILGRSETQECLFYNANWELDRTNQTGVEPCEGEKDKRLHCFATWRNISGSIEIVKKGCWLDDFNCYDRTDCVETKENPQVYFCCCEGNMCNEKFSYFPEMEVTQPTS

SEQ ID NO: 26 - protein, 109 aa, synthetic construct
  source 1..109: note = Synthetic Construct
GAILGRSETQECLFYNANWELDRTNQTGVEPCEGEKDKRLHCFATWRNISGSIEIVKKGCWLDDINCYDRTDCVETEENPQVYFCCCEGNMCNEKFSYFPEMEVTQPTS

SEQ ID NO: 27 - protein, 109 aa, synthetic construct
  source 1..109: note = Synthetic Construct
GAILGRSETQECLFYNANWELDRTNQTGVEPCEGEKDKRLHCFATWKNISGSIEIVKKGCWLDDFNCYDRTDCVETEENPQVYFCCCEGNMCNEKFSYFPEMEVTQPTS

SEQ ID NO: 28 - protein, 109 aa, synthetic construct
  source 1..109: note = Synthetic Construct
GAILGRSETQECLFYNANWELERTNQTGVERCEGEKDKRLHCYATWKNISGSIEIVKKGCWLDDINCYDRTDCVETKENPQVYFCCCEGNMCNEKFSYFPEMEVTQPTS

SEQ ID NO: 29 - protein, 109 aa, synthetic construct
  source 1..109: note = Synthetic Construct
GAILGRSETQECLFYNANWELERTNQTGVERCEGEKDKRLHCFATWRNISGSIEIVKKGCWLDDINCYDRTDCVETKENPQVYFCCCEGNMCNEKFSYFPEMEVTQPTS

SEQ ID NO: 30 - protein, 109 aa, synthetic construct
  source 1..109: note = Synthetic Construct
GAILGRSETQECLFYNANWELERTNQTGVERCEGEKDKRLHCFATWKNISGSIEIVKKGCWLDDFNCYDRTDCVETKENPQVYFCCCEGNMCNEKFSYFPEMEVTQPTS

SEQ ID NO: 31 - protein, 109 aa, synthetic construct
  source 1..109: note = Synthetic Construct
GAILGRSETQECLFYNANWELERTNQTGVERCEGEKDKRLHCFATWKNISGSIEIVKKGCWLDDINCYDRTDCVETEENPQVYFCCCEGNMCNEKFSYFPEMEVTQPTS

SEQ ID NO: 32 - protein, 109 aa, synthetic construct
  source 1..109: note = Synthetic Construct
GAILGRSETQECLFYNANWELERTNQTGVEPCEGEKDKRLHCYATWRNISGSIEIVKKGCWLDDINCYDRTDCVETKENPQVYFCCCEGNMCNEKFSYFPEMEVTQPTS

SEQ ID NO: 33 - protein, 109 aa, synthetic construct
  source 1..109: note = Synthetic Construct
GAILGRSETQECLFYNANWELERTNQTGVEPCEGEKDKRLHCYATWKNISGSIEIVKKGCWLDDFNCYDRTDCVETKENPQVYFCCCEGNMCNEKFSYFPEMEVTQPTS

SEQ ID NO: 34 - protein, 109 aa, synthetic construct
  source 1..109: note = Synthetic Construct
GAILGRSETQECLFYNANWELERTNQTGVEPCEGEKDKRLHCYATWKNISGSIEIVKKGCWLDDINCYDRTDCVETEENPQVYFCCCEGNMCNEKFSYFPEMEVTQPTS

SEQ ID NO: 35 - protein, 109 aa, synthetic construct
  source 1..109: note = Synthetic Construct
GAILGRSETQECLFYNANWELERTNQTGVEPCEGEKDKRLHCFATWRNISGSIEIVKKGCWLDDFNCYDRTDCVETKENPQVYFCCCEGNMCNEKFSYFPEMEVTQPTS

SEQ ID NO: 36 - protein, 109 aa, synthetic construct
  source 1..109: note = Synthetic Construct
GAILGRSETQECLFYNANWELERTNQTGVEPCEGEKDKRLHCFATWRNISGSIEIVKKGCWLDDINCYDRTDCVETEENPQVYFCCCEGNMCNEKFSYFPEMEVTQPTS

SEQ ID NO: 37 - protein, 109 aa, synthetic construct
  source 1..109: note = Synthetic Construct
GAILGRSETQECLFYNANWELERTNQTGVEPCEGEKDKRLHCFATWKNISGSIEIVKKGCWLDDFNCYDRTDCVETEENPQVYFCCCEGNMCNEKFSYFPEMEVTQPTS

SEQ ID NO: 38 - protein, 109 aa, synthetic construct
  source 1..109: note = Synthetic Construct
GAILGRSETQECLFYNANWELDRTNQTGVERCEGEKDKRLHCYATWRNISGSIEIVKKGCWLDDINCYDRTDCVETKENPQVYFCCCEGNMCNEKFSYFPEMEVTQPTS

SEQ ID NO: 39 - protein, 109 aa, synthetic construct
  source 1..109: note = Synthetic Construct
GAILGRSETQECLFYNANWELDRTNQTGVERCEGEKDKRLHCYATWKNISGSIEIVKKGCWLDDFNCYDRTDCVETKENPQVYFCCCEGNMCNEKFSYFPEMEVTQPTS

SEQ ID NO: 40 - protein, 109 aa, synthetic construct
  source 1..109: note = Synthetic Construct
GAILGRSETQECLFYNANWELDRTNQTGVERCEGEKDKRLHCYATWKNISGSIEIVKKGCWLDDINCYDRTDCVETEENPQVYFCCCEGNMCNEKFSYFPEMEVTQPTS

SEQ ID NO: 41 - protein, 109 aa, synthetic construct
  source 1..109: note = Synthetic Construct
GAILGRSETQECLFYNANWELDRTNQTGVERCEGEKDKRLHCFATWRNISGSIEIVKKGCWLDDFNCYDRTDCVETKENPQVYFCCCEGNMCNEKFSYFPEMEVTQPTS

SEQ ID NO: 42 - protein, 109 aa, synthetic construct
  source 1..109: note = Synthetic Construct
GAILGRSETQECLFYNANWELDRTNQTGVERCEGEKDKRLHCFATWRNISGSIEIVKKGCWLDDINCYDRTDCVETEENPQVYFCCCEGNMCNEKFSYFPEMEVTQPTS

SEQ ID NO: 43 - protein, 109 aa, synthetic construct
  source 1..109: note = Synthetic Construct
GAILGRSETQECLFYNANWELDRTNQTGVERCEGEKDKRLHCFATWKNISGSIEIVKKGCWLDDFNCYDRTDCVETEENPQVYFCCCEGNMCNEKFSYFPEMEVTQPTS

SEQ ID NO: 44 - protein, 109 aa, synthetic construct
  source 1..109: note = Synthetic Construct
GAILGRSETQECLFYNANWELDRTNQTGVEPCEGEKDKRLHCYATWRNISGSIEIVKKGCWLDDFNCYDRTDCVETKENPQVYFCCCEGNMCNEKFSYFPEMEVTQPTS

SEQ ID NO: 45 - protein, 109 aa, synthetic construct
  source 1..109: note = Synthetic Construct
GAILGRSETQECLFYNANWELDRTNQTGVEPCEGEKDKRLHCYATWRNISGSIEIVKKGCWLDDINCYDRTDCVETEENPQVYFCCCEGNMCNEKFSYFPEMEVTQPTS

SEQ ID NO: 46 - protein, 109 aa, synthetic construct
  source 1..109: note = Synthetic Construct
GAILGRSETQECLFYNANWELDRTNQTGVEPCEGEKDKRLHCYATWKNISGSIEIVKKGCWLDDFNCYDRTDCVETEENPQVYFCCCEGNMCNEKFSYFPEMEVTQPTS

SEQ ID NO: 47 - protein, 109 aa, synthetic construct
  source 1..109: note = Synthetic Construct
GAILGRSETQECLFYNANWELDRTNQTGVEPCEGEKDKRLHCFATWRNISGSIEIVKKGCWLDDFNCYDRTDCVETEENPQVYFCCCEGNMCNEKFSYFPEMEVTQPTS

SEQ ID NO: 48 - protein, 109 aa, synthetic construct
  source 1..109: note = Synthetic Construct
GAILGRSETQECLFYNANWELERTNQTGVERCEGEKDKRLHCYATWRNISGSIEIVKKGCWLDDINCYDRTDCVETKENPQVYFCCCEGNMCNEKFSYFPEMEVTQPTS

SEQ ID NO: 49 - protein, 109 aa, synthetic construct
  source 1..109: note = Synthetic Construct
GAILGRSETQECLFYNANWELERTNQTGVERCEGEKDKRLHCYATWKNISGSIEIVKKGCWLDDFNCYDRTDCVETKENPQVYFCCCEGNMCNEKFSYFPEMEVTQPTS

SEQ ID NO: 50 - protein, 109 aa, synthetic construct
  source 1..109: note = Synthetic Construct
GAILGRSETQECLFYNANWELERTNQTGVERCEGEKDKRLHCYATWKNISGSIEIVKKGCWLDDINCYDRTDCVETEENPQVYFCCCEGNMCNEKFSYFPEMEVTQPTS

SEQ ID NO: 51 - protein, 109 aa, synthetic construct
  source 1..109: note = Synthetic Construct
GAILGRSETQECLFYNANWELERTNQTGVERCEGEKDKRLHCFATWRNISGSIEIVKKGCWLDDFNCYDRTDCVETKENPQVYFCCCEGNMCNEKFSYFPEMEVTQPTS

SEQ ID NO: 52 - protein, 109 aa, synthetic construct
  source 1..109: note = Synthetic Construct
GAILGRSETQECLFYNANWELERTNQTGVERCEGEKDKRLHCFATWRNISGSIEIVKKGCWLDDINCYDRTDCVETEENPQVYFCCCEGNMCNEKFSYFPEMEVTQPTS

SEQ ID NO: 53 - protein, 109 aa, synthetic construct
  source 1..109: note = Synthetic Construct
GAILGRSETQECLFYNANWELERTNQTGVERCEGEKDKRLHCFATWKNISGSIEIVKKGCWLDDFNCYDRTDCVETEENPQVYFCCCEGNMCNEKFSYFPEMEVTQPTS

SEQ ID NO: 54 - protein, 109 aa, synthetic construct
  source 1..109: note = Synthetic Construct
GAILGRSETQECLFYNANWELERTNQTGVEPCEGEKDKRLHCYATWRNISGSIEIVKKGCWLDDFNCYDRTDCVETKENPQVYFCCCEGNMCNEKFSYFPEMEVTQPTS

SEQ ID NO: 55 - protein, 109 aa, synthetic construct
  source 1..109: note = Synthetic Construct
GAILGRSETQECLFYNANWELERTNQTGVEPCEGEKDKRLHCYATWRNISGSIEIVKKGCWLDDINCYDRTDCVETEENPQVYFCCCEGNMCNEKFSYFPEMEVTQPTS

SEQ ID NO: 56 - protein, 109 aa, synthetic construct
  source 1..109: note = Synthetic Construct
GAILGRSETQECLFYNANWELERTNQTGVEPCEGEKDKRLHCYATWKNISGSIEIVKKGCWLDDFNCYDRTDCVETEENPQVYFCCCEGNMCNEKFSYFPEMEVTQPTS

SEQ ID NO: 57 - protein, 109 aa, synthetic construct
  source 1..109: note = Synthetic Construct
GAILGRSETQECLFYNANWELERTNQTGVEPCEGEKDKRLHCFATWRNISGSIEIVKKGCWLDDFNCYDRTDCVETEENPQVYFCCCEGNMCNEKFSYFPEMEVTQPTS

SEQ ID NO: 58 - protein, 109 aa, synthetic construct
  source 1..109: note = Synthetic Construct
GAILGRSETQECLFYNANWELDRTNQTGVERCEGEKDKRLHCYATWRNISGSIEIVKKGCWLDDFNCYDRTDCVETKENPQVYFCCCEGNMCNEKFSYFPEMEVTQPTS

SEQ ID NO: 59 - protein, 109 aa, synthetic construct
  source 1..109: note = Synthetic Construct
GAILGRSETQECLFYNANWELDRTNQTGVERCEGEKDKRLHCYATWRNISGSIEIVKKGCWLDDINCYDRTDCVETEENPQVYFCCCEGNMCNEKFSYFPEMEVTQPTS

SEQ ID NO: 60 - protein, 109 aa, synthetic construct
  source 1..109: note = Synthetic Construct
GAILGRSETQECLFYNANWELDRTNQTGVERCEGEKDKRLHCYATWKNISGSIEIVKKGCWLDDFNCYDRTDCVETEENPQVYFCCCEGNMCNEKFSYFPEMEVTQPTS

SEQ ID NO: 61 - protein, 109 aa, synthetic construct
  source 1..109: note = Synthetic Construct
GAILGRSETQECLFYNANWELDRTNQTGVERCEGEKDKRLHCFATWRNISGSIEIVKKGCWLDDFNCYDRTDCVETEENPQVYFCCCEGNMCNEKFSYFPEMEVTQPTS

SEQ ID NO: 62 - protein, 109 aa, synthetic construct
  source 1..109: note = Synthetic Construct
GAILGRSETQECLFYNANWELDRTNQTGVEPCEGEKDKRLHCYATWRNISGSIEIVKKGCWLDDFNCYDRTDCVETEENPQVYFCCCEGNMCNEKFSYFPEMEVTQPTS

SEQ ID NO: 63 - protein, 109 aa, synthetic construct
  source 1..109: note = Synthetic Construct
GAILGRSETQECLFYNANWELERTNQTGVERCEGEKDKRLHCYATWRNISGSIEIVKKGCWLDDFNCYDRTDCVETKENPQVYFCCCEGNMCNEKFSYFPEMEVTQPTS

SEQ ID NO: 64 - protein, 109 aa, synthetic construct
  source 1..109: note = Synthetic Construct
GAILGRSETQECLFYNANWELERTNQTGVERCEGEKDKRLHCYATWRNISGSIEIVKKGCWLDDINCYDRTDCVETEENPQVYFCCCEGNMCNEKFSYFPEMEVTQPTS

SEQ ID NO: 65 - protein, 109 aa, synthetic construct
  source 1..109: note = Synthetic Construct
GAILGRSETQECLFYNANWELERTNQTGVERCEGEKDKRLHCYATWKNISGSIEIVKKGCWLDDFNCYDRTDCVETEENPQVYFCCCEGNMCNEKFSYFPEMEVTQPTS

SEQ ID NO: 66 - protein, 109 aa, synthetic construct
  source 1..109: note = Synthetic Construct
GAILGRSETQECLFYNANWELERTNQTGVERCEGEKDKRLHCFATWRNISGSIEIVKKGCWLDDFNCYDRTDCVETEENPQVYFCCCEGNMCNEKFSYFPEMEVTQPTS

SEQ ID NO: 67 - protein, 109 aa, synthetic construct
  source 1..109: note = Synthetic Construct
GAILGRSETQECLFYNANWELDRTNQTGVERCEGEKDKRLHCYATWRNISGSIEIVKKGCWLDDFNCYDRTDCVETEENPQVYFCCCEGNMCNEKFSYFPEMEVTQPTS

SEQ ID NO: 68 - protein, 109 aa, synthetic construct
  source 1..109: note = Synthetic Construct
GAILGRSETQECLFYNANWELERTNQTGVEPCEGEKDKRLHCYATWRNISGSIEIVKKGCWLDDFNCYDRTDCVETEENPQVYFCCCEGNMCNEKFSYFPEMEVTQPTS

SEQ ID NO: 69 - protein, 109 aa, synthetic construct
  source 1..109: note = Synthetic Construct
GAILGRSETQECLFYNANWELERTNQTGVERCEGEKDKRLHCYATWRNISGSIEIVKKGCWLDDFNCYDRTDCVETEENPQVYFCCCEGNMCNEKFSYFPEMEVTQPTS

SEQ ID NO: 70 - protein, 109 aa, synthetic construct
  source 1..109: note = Synthetic Construct
GAILGRSETQECLYYNANWELERTNQTGVERCEGEQDKRLHCYATWRNISGSIEIVKKGCWLDDFNCYDRTDCVETEENPQVYFCCCEGNMCNEKFSYFPEMEVTQPTS

SEQ ID NO: 71 - protein, 111 aa, synthetic construct
  source 1..111: note = Synthetic Construct
GAILGRSETQECLFYNANWELERTNQTGVERCEGEKDKRLHCYATWRNISGSIEIVKKGCWLDDFNCYDRTDCVETEENPQVYFCCCEGNMCNEKFSYFPEMEVTQPTSNP

SEQ ID NO: 72 - protein, 115 aa, synthetic construct
  source 1..115: note = Synthetic Construct
GAILGRSETQECLFYNANWELERTNQTGVERCEGEKDKRLHCYATWRNISGSIEIVKKGCWLDDFNCYDRTDCVETEENPQVYFCCCEGNMCNEKFSYFPEMEVTQPTSNPVTPK

SEQ ID NO: 73 - protein, 109 aa, Homo sapiens
GAILGRSETQECLFFNANWEKDRTNQTGVEPCYGDKDKRRHCFATWKNISGSIEIVKQGCWLDDINCYDRTDCVEKKDSPEVYFCCCEGNMCNEKFSYFPEMEVTQPTS

SEQ ID NO: 74 - protein, 115 aa, Homo sapiens
GRGEAETRECIYYNANWELERTNQSGLERCEGEQDKRLHCYASWRNSSGTIELVKKGCWLDDFNCYDRQECVATEENPQVYFCCCEGNFCNERFTHLPEAGGPEVTYEPPPTAPT

SEQ ID NO: 75 - protein, 513 aa, Homo sapiens
MGAAAKLAFAVFLISCSSGAILGRSETQECLFFNANWEKDRTNQTGVEPCYGDKDKRRHCFATWKNISGSIEIVKQGCWLDDINCYDRTDCVEKKDSPEVYFCCCEGNMCNEKFSYFPEMEVTQPTSNPVTPKPPYYNILLYSLVPLMLIAGIVICAFWVYRHHKMAYPPVLVPTQDPGPPPPSPLLGLKPLQLLEVKARGRFGCVWKAQLLNEYVAVKIFPIQDKQSWQNEYEVYSLPGMKHENILQFIGAEKRGTSVDVDLWLITAFHEKGSLSDFLKANVVSWNELCHIAETMARGLAYLHEDIPGLKDGHKPAISHRDIKSKNVLLKNNLTACIADFGLALKFEAGKSAGDTHGQVGTRRYMAPEVLEGAINFQRDAFLRIDMYAMGLVLWELASRCTAADGPVDEYMLPFEEEIGQHPSLEDMQEVVVHKKKRPVLRDYWQKHAGMAMLCETIEECWDHDAEARLSAGCVGERITQMQRLTNIITTEDIVTVVTMVTNVDFPPKESSL

SEQ ID NO: 76 - protein, 109 aa, synthetic construct
  source 1..109: note = Synthetic Construct
GAILGRSETQECLFFNANWEKDRTNQTGVEPCYGDKDKRRHCFATWANISGSIEIVKQGCWLDDINCYDRTDCVEKKDSPEVYFCCCEGNMCNEKFSYFPEMEVTQPTS

SEQ ID NO: 77 - protein, 109 aa, synthetic construct
  source 1..109: note = Synthetic Construct
GAILGRSETQECLFFNANWAKDRTNQTGVEPCYGDKDKRRHCFATWKNISGSIEIVKQGCWLDDINCYDRTDCVEKKDSPEVYFCCCEGNMCNEKFSYFPEMEVTQPTS

SEQ ID NO: 78 - protein, 109 aa, synthetic construct
  source 1..109: note = Synthetic Construct
GAILGRSETQECLFFNANWEKDATNQTGVEPCYGDKDKRRHCFATWKNISGSIEIVKQGCWLDDINCYDRTDCVEKKDSPEVYFCCCEGNMCNEKFSYFPEMEVTQPTS

SEQ ID NO: 79 - protein, 109 aa, synthetic construct
  source 1..109: note = Synthetic Construct
GAILGRSETQECLFFNANWEKDRTNQTGVEPCYGDKAKRRHCFATWKNISGSIEIVKQGCWLDDINCYDRTDCVEKKDSPEVYFCCCEGNMCNEKFSYFPEMEVTQPTS

SEQ ID NO: 80 - protein, 109 aa, synthetic construct
  source 1..109: note = Synthetic Construct
GAILGRSETQECLFFNANWEKDRTNQTGVEPCYGDKDARRHCFATWKNISGSIEIVKQGCWLDDINCYDRTDCVEKKDSPEVYFCCCEGNMCNEKFSYFPEMEVTQPTS

SEQ ID NO: 81 - protein, 109 aa, synthetic construct
  source 1..109: note = Synthetic Construct
GAILGRSETQECLFFNANWEKDRTNQTGVEPCYGDKDKARHCFATWKNISGSIEIVKQGCWLDDINCYDRTDCVEKKDSPEVYFCCCEGNMCNEKFSYFPEMEVTQPTS

SEQ ID NO: 82 - protein, 109 aa, synthetic construct
  source 1..109: note = Synthetic Construct
GAILGRSETQECLFFNANWEKDRTNQTGVEPCYGDKDKRRHCFATWKNISGSIEIVAQGCWLDDINCYDRTDCVEKKDSPEVYFCCCEGNMCNEKFSYFPEMEVTQPTS

SEQ ID NO: 83 - protein, 109 aa, synthetic construct
  source 1..109: note = Synthetic Construct
GAILGRSETQECLFFNANWEKDRTNQTGVEPCYGDKDKRRHCFATWKNISGSIEIVYQGCWLDDINCYDRTDCVEKKDSPEVYFCCCEGNMCNEKFSYFPEMEVTQPTS

SEQ ID NO: 84 - protein, 109 aa, synthetic construct
  source 1..109: note = Synthetic Construct
GAILGRSETQECLFFNANWEKDRTNQTGVEPCYGDKDKRRHCFATWKNISGSIEIVFQGCWLDDINCYDRTDCVEKKDSPEVYFCCCEGNMCNEKFSYFPEMEVTQPTS

SEQ ID NO: 85 - protein, 109 aa, synthetic construct
  source 1..109: note = Synthetic Construct
GAILGRSETQECLFFNANWEKDRTNQTGVEPCYGDKDKRRHCFATWKNISGSIEIVIQGCWLDDINCYDRTDCVEKKDSPEVYFCCCEGNMCNEKFSYFPEMEVTQPTS

SEQ ID NO: 86 - protein, 109 aa, synthetic construct
  source 1..109: note = Synthetic Construct
GAILGRSETQECLFFNANWEKDRTNQTGVEPCYGDKDKRRHCFATWKNISGSIEIVKQGCALDDINCYDRTDCVEKKDSPEVYFCCCEGNMCNEKFSYFPEMEVTQPTS

SEQ ID NO: 87 - protein, 109 aa, synthetic construct
  source 1..109: note = Synthetic Construct
GAILGRSETQECLFFNANWEKDRTNQTGVEPCYGDKDKRRHCFATWKNISGSIEIVKQGCWADDINCYDRTDCVEKKDSPEVYFCCCEGNMCNEKFSYFPEMEVTQPTS

SEQ ID NO: 88 - protein, 109 aa, synthetic construct
  source 1..109: note = Synthetic Construct
GAILGRSETQECLFFNANWEKDRTNQTGVEPCYGDKDKRRHCFATWKNISGSIEIVKQGCWLKDINCYDRTDCVEKKDSPEVYFCCCEGNMCNEKFSYFPEMEVTQPTS

SEQ ID NO: 89 - protein, 109 aa, synthetic construct
  source 1..109: note = Synthetic Construct
GAILGRSETQECLFFNANWEKDRTNQTGVEPCYGDKDKRRHCFATWKNISGSIEIVKQGCWLRDINCYDRTDCVEKKDSPEVYFCCCEGNMCNEKFSYFPEMEVTQPTS

SEQ ID NO: 90 - protein, 109 aa, synthetic construct
  source 1..109: note = Synthetic Construct
GAILGRSETQECLFFNANWEKDRTNQTGVEPCYGDKDKRRHCFATWKNISGSIEIVKQGCWLADINCYDRTDCVEKKDSPEVYFCCCEGNMCNEKFSYFPEMEVTQPTS

SEQ ID NO: 91 - protein, 109 aa, synthetic construct
  source 1..109: note = Synthetic Construct
GAILGRSETQECLFFNANWEKDRTNQTGVEPCYGDKDKRRHCFATWKNISGSIEIVKQGCWLFDINCYDRTDCVEKKDSPEVYFCCCEGNMCNEKFSYFPEMEVTQPTS

SEQ ID NO: 92 - protein, 109 aa, synthetic construct
  source 1..109: note = Synthetic Construct
GAILGRSETQECLFFNANWEKDRTNQTGVEPCYGDKDKRRHCFATWKNISGSIEIVKQGCWLGDINCYDRTDCVEKKDSPEVYFCCCEGNMCNEKFSYFPEMEVTQPTS

SEQ ID NO: 93 - protein, 109 aa, synthetic construct
  source 1..109: note = Synthetic Construct
GAILGRSETQECLFFNANWEKDRTNQTGVEPCYGDKDKRRHCFATWKNISGSIEIVKQGCWLMDINCYDRTDCVEKKDSPEVYFCCCEGNMCNEKFSYFPEMEVTQPTS

SEQ ID NO: 94 - protein, 109 aa, synthetic construct
  source 1..109: note = Synthetic Construct
GAILGRSETQECLFFNANWEKDRTNQTGVEPCYGDKDKRRHCFATWKNISGSIEIVKQGCWLNDINCYDRTDCVEKKDSPEVYFCCCEGNMCNEKFSYFPEMEVTQPTS

SEQ ID NO: 95 - protein, 109 aa, synthetic construct
  source 1..109: note = Synthetic Construct
GAILGRSETQECLFFNANWEKDRTNQTGVEPCYGDKDKRRHCFATWKNISGSIEIVKQGCWLIDINCYDRTDCVEKKDSPEVYFCCCEGNMCNEKFSYFPEMEVTQPTS

SEQ ID NO: 96 - protein, 109 aa, synthetic construct
  source 1..109: note = Synthetic Construct
GAILGRSETQECLFFNANWEKDRTNQTGVEPCYGDKDKRRHCFATWKNISGSIEIVKQGCWLDDANCYDRTDCVEKKDSPEVYFCCCEGNMCNEKFSYFPEMEVTQPTS

SEQ ID NO: 97 - protein, 225 aa, Homo sapiens
THTCPPCPAPELLGGPSVFLFPPKPKDTLMISRTPEVTCVVVDVSHEDPEVKFNWYVDGVEVHNAKTKPREEQYNSTYRVVSVLTVLHQDWLNGKEYKCKVSNKALPVPIEKTISKAKGQPREPQVYTLPPSREEMTKNQVSLTCLVKGFYPSDIAVEWESNGQPENNYKTTPPVLDSDGPFFLYSKLTVDKSRWQQGNVFSCSVMHEALHNHYTQKSLSLSPGK

SEQ ID NO: 98 - protein, 4 aa, synthetic construct
  source 1..4: note = Synthetic Construct
GGGA

SEQ ID NO: 99 - protein, 4 aa, synthetic construct
  source 1..4: note = Synthetic Construct
GGGS

SEQ ID NO: 100 - protein, 4 aa, synthetic construct
  source 1..4: note = Synthetic Construct
GGGG

SEQ ID NO: 101 - protein, 5 aa, synthetic construct
  source 1..5: note = Synthetic Construct
GGGGA

SEQ ID NO: 102 - protein, 5 aa, synthetic construct
  source 1..5: note = Synthetic Construct
GGGGS

SEQ ID NO: 103 - protein, 5 aa, synthetic construct
  source 1..5: note = Synthetic Construct
GGGGG

SEQ ID NO: 104 - protein, 4 aa, synthetic construct
  source 1..4: note = Synthetic Construct
GGAG

SEQ ID NO: 105 - protein, 4 aa, synthetic construct
  source 1..4: note = Synthetic Construct
GGSG

SEQ ID NO: 106 - protein, 4 aa, synthetic construct
  source 1..4: note = Synthetic Construct
AGGG

SEQ ID NO: 107 - protein, 4 aa, synthetic construct
  source 1..4: note = Synthetic Construct
SGGG

SEQ ID NO: 108 - protein, 4 aa, synthetic construct
  source 1..4: note = Synthetic Construct
GAGA

SEQ ID NO: 109 - protein, 4 aa, synthetic construct
  source 1..4: note = Synthetic Construct
GSGS

SEQ ID NO: 110 - protein, 6 aa, synthetic construct
  source 1..6: note = Synthetic Construct
GAGAGA

SEQ ID NO: 111 - protein, 6 aa, synthetic construct
  source 1..6: note = Synthetic Construct
GSGSGS

SEQ ID NO: 112 - protein, 8 aa, synthetic construct
  source 1..8: note = Synthetic Construct
GAGAGAGA

SEQ ID NO: 113 - protein, 8 aa, synthetic construct
  source 1..8: note = Synthetic Construct
GSGSGSGS

SEQ ID NO: 114 - protein, 10 aa, synthetic construct
  source 1..10: note = Synthetic Construct
GAGAGAGAGA

SEQ ID NO: 115 - protein, 10 aa, synthetic construct
  source 1..10: note = Synthetic Construct
GSGSGSGSGS

SEQ ID NO: 116 - protein, 12 aa, synthetic construct
  source 1..12: note = Synthetic Construct
GAGAGAGAGAGA

SEQ ID NO: 117 - protein, 12 aa, synthetic construct
  source 1..12: note = Synthetic Construct
GSGSGSGSGSGS

SEQ ID NO: 118 - protein, 6 aa, synthetic construct
  source 1..6: note = Synthetic Construct
GGAGGA

SEQ ID NO: 119 - protein, 6 aa, synthetic construct
  source 1..6: note = Synthetic Construct
GGSGGS

SEQ ID NO: 120 - protein, 9 aa, synthetic construct
  source 1..9: note = Synthetic Construct
GGAGGAGGA

SEQ ID NO: 121 - protein, 9 aa, synthetic construct
  source 1..9: note = Synthetic Construct
GGSGGSGGS

SEQ ID NO: 122 - protein, 12 aa, synthetic construct
  source 1..12: note = Synthetic Construct
GGAGGAGGAGGA

SEQ ID NO: 123 - protein, 12 aa, synthetic construct
  source 1..12: note = Synthetic Construct
GGSGGSGGSGGS

SEQ ID NO: 124 - protein, 8 aa, synthetic construct
  source 1..8: note = Synthetic Construct
GGAGGGAG

SEQ ID NO: 125 - protein, 8 aa, synthetic construct
  source 1..8: note = Synthetic Construct
GGSGGGSG

SEQ ID NO: 126 - protein, 12 aa, synthetic construct
  source 1..12: note = Synthetic Construct
GGAGGGAGGGAG

SEQ ID NO: 127 - protein, 12 aa, synthetic construct
  source 1..12: note = Synthetic Construct
GGSGGGSGGGSG

SEQ ID NO: 128 - protein, 15 aa, synthetic construct
  source 1..15: note = Synthetic Construct
GGGGAGGGGAGGGGA

SEQ ID NO: 129 - protein, 15 aa, synthetic construct
  source 1..15: note = Synthetic Construct
GGGGSGGGGSGGGGS

SEQ ID NO: 130 - protein, 5 aa, synthetic construct
  source 1..5: note = Synthetic Construct
GGGAG

SEQ ID NO: 131 - protein, 6 aa, synthetic construct
  source 1..6: note = Synthetic Construct
GGGAGG

SEQ ID NO: 132 - protein, 7 aa, synthetic construct
  source 1..7: note = Synthetic Construct
GGGAGGG

SEQ ID NO: 133 - protein, 4 aa, synthetic construct
  source 1..4: note = Synthetic Construct
AAAL

SEQ ID NO: 134 - protein, 4 aa, synthetic construct
  source 1..4: note = Synthetic Construct
AAAK

SEQ ID NO: 135 - protein, 4 aa, synthetic construct
  source 1..4: note = Synthetic Construct
AAAR

SEQ ID NO: 136 - protein, 14 aa, synthetic construct
  source 1..14: note = Synthetic Construct
EGKSSGSGSESKST

SEQ ID NO: 137 - protein, 12 aa, synthetic construct
  source 1..12: note = Synthetic Construct
GSAGSAAGSGEF

SEQ ID NO: 138 - protein, 12 aa, synthetic construct
  source 1..12: note = Synthetic Construct
AEAAAKEAAAKA

SEQ ID NO: 139 - protein, 18 aa, synthetic construct
  source 1..18: note = Synthetic Construct
KESGSVSSEQLAQFRSLD

SEQ ID NO: 140 - protein, 10 aa, synthetic construct
  source 1..10: note = Synthetic Construct
GENLYFQSGG

SEQ ID NO: 141 - protein, 8 aa, synthetic construct
  source 1..8: note = Synthetic Construct
SACYCELS

SEQ ID NO: 142 - protein, 5 aa, synthetic construct
  source 1..5: note = Synthetic Construct
RSIAT

SEQ ID NO: 143 - protein, 17 aa, synthetic construct
  source 1..17: note = Synthetic Construct
RPACKIPNDLKQKVMNH

SEQ ID NO: 144 - protein, 36 aa, synthetic construct
  source 1..36: note = Synthetic Construct
GGSAGGSGSGSSGGSSGASGTGTAGGTGSGSGTGSG

SEQ ID NO: 145 - protein, 17 aa, synthetic construct
  source 1..17: note = Synthetic Construct
AAANSSIDLISVPVDSR

SEQ ID NO: 146 - protein, 36 aa, synthetic construct
  source 1..36: note = Synthetic Construct
GGSGGGSEGGGSEGGGSEGGGSEGGGSEGGGSGGGS

SEQ ID NO: 147 - protein, 5 aa, synthetic construct
  source 1..5: note = Synthetic Construct
EAAAK

SEQ ID NO: 148 - protein, 5 aa, synthetic construct
  source 1..5: note = Synthetic Construct
PAPAP

SEQ ID NO: 149 - protein, 115 aa, synthetic construct
  source 1..115: note = Synthetic Construct
GRGEAETRECIFYNANWEKDRTNQSGLEPCYGDQDKRRHCFASWKNSSGTIELVKQGCWLDDINCYDRQECVAKKDSPEVYFCCCEGNFCNERFTHLPEAGGPEVTYEPPPTAPT

SEQ ID NO: 150 - protein, 109 aa, synthetic construct
  source 1..109: note = Synthetic Construct
GAILGRSETQECLFYNANWELERTNQTGVERCEGEKDKRLHCYATWRNISGSIEIVAKGCWLDDFNCYDRTDCVETEENPQVYFCCCEGNMCNEKFSYFPEMEVTQPTS

SEQ ID NO: 151 - protein, 246 aa, Homo sapiens
MEWSWVFLFFLSVTTGVHSDKTHTCPPCPAPELLGGPSVFLFPPKPKDTLMISRTPEVTCVVVDVSHEDPEVKFNWYVDGVEVHNAKTKPREEQYNSTYRVVSVLTVLHQDWLNGKEYKCKVSNKALPAPIEKTISKAKGQPREPQVYTLPPSRDELTKNQVSLTCLVKGFYPSDIAVEWESNGQPENNYKTTPPVLDSDGSFFLYSKLTVDKSRWQQGNVFSCSVMHEALHNHYTQKSLSLSPGK

SEQ ID NO: 152 - protein, 11 aa, synthetic construct
  source 1..11: note = Synthetic Construct
DICLPRWGCLW

SEQ ID NO: 153 - protein, 93 aa, Homo sapiens
GPVEVFITETPSQPNSHPIQWNAPQPSHISKYILRWRPKNSVGRWKEATIPGHLNSYTIKGLKPGVVYEGQLISIQQYGHQEVTRFDFTTTST

SEQ ID NO: 154 - protein, 609 aa, Homo sapiens [sequence omitted]

SEQ ID NO: 155 - protein, 6 aa, Homo sapiens
NPVTPK

SEQ ID NO: 156 - protein, 4 aa, Homo sapiens
TEEN

SEQ ID NO: 157 - protein, 4 aa, synthetic construct
  source 1..4: note = Synthetic Construct
TKEN

SEQ ID NO: 158 - protein, 4 aa, Homo sapiens
VTPK

SEQ ID NO: 159 - protein, 10 aa, synthetic construct
  VARIANT 1: note = Any amino acid
  VARIANT 3: note = Any amino acid
  VARIANT 5: note = Any amino acid
  VARIANT 7: note = Any amino acid
  VARIANT 9: note = Any amino acid
  VARIANT 1..10: note = This sequence may encompass 1-5 XP repeating units
XPXPXPXPXP

SEQ ID NO: 160 - protein, 81 aa, Homo sapiens
CLFFNANWEKDRTNQTGVEPCYGDKDKRRHCFATWKNISGSIEIVKQGCWLDDINCYDRTDCVEKKDSPEVYFCCCEGNMC

SEQ ID NO: 161 - protein, 81 aa, Homo sapiens
CIYYNANWELERTNQSGLERCEGEQDKRLHCYASWRNSSGTIELVKKGCWLDDFNCYDRQECVATEENPQVYFCCCEGNFC